European Patent Specification EP 3 873 526 B1, published September 4, 2024. Title: Anti-rabies monoclonal antibodies and cocktail thereof. Applicant: Cadila Healthcare Limited. The sequence listing filed with the application follows.

SEQUENCE LISTING (12 sequences)

SEQ ID NO: 1 - protein, 5 aa, Murine monoclonal antibody (CDRH1 of mAb A)
SSWMH

SEQ ID NO: 2 - protein, 17 aa, Murine monoclonal antibody (CDRH2 of mAb A)
QTHPNSGYTNYNEKFKG

SEQ ID NO: 3 - protein, 12 aa, Murine monoclonal antibody (CDRH3 of mAb A)
ESGDGPHWYFDV

SEQ ID NO: 4 - protein, 11 aa, Murine monoclonal antibody (CDRL1 of mAb A)
KASQDVSTAVA

SEQ ID NO: 5 - protein, 7 aa, Murine monoclonal antibody  (CDRL2 of mAb A)
SASYRYT

SEQ ID NO: 6 - protein, 9 aa, Murine monoclonal antibody (CDRL3 of mAb A)
QQHYSSPHT

SEQ ID NO: 7 - protein, 121 aa, Murine monoclonal antibody (HCVR of mAb A)
QVQLQQPGSVLVRPGASVKLSCKTSGYAFTSSWMHWAKQRPGQGLEWIGQTHPNSGYTNYNEKFKGKATLTVDTSSSTAYVDLSSLTSEDSAVYYCARESGDGPHWYFDVWGAGTAVTVSS

SEQ ID NO: 8 - protein, 107 aa, Murine monoclonal antibody (HCVR of mAb A) (LCVR of mAb A)
DIVMTQSHKFMSTSVGDRVSITCKASQDVSTAVAWYQQKPGQSPKLLIYSASYRYTGVPDRFTGSGSGTDFTFTISSVQAEDLAVYYCQQHYSSPHTFGGGTKLETK

SEQ ID NO: 9 - protein, 445 aa, Murine monoclonal antibody (HC of mAb A)
QVQLQQPGSVLVRPGASVKLSCKTSGYAFTSSWMHWAKQRPGQGLEWIGQTHPNSGYTNYNEKFKGKATLTVDTSSSTAYVDLSSLTSEDSAVYYCARESGDGPHWYFDVWGAGTAVTVSSAKTTPPSVYPLAPGSAAQTNSMVTLGCLVKGYFPEPVTVTWNSGSLSSGVHTFPAVLQSDLYTLSSSVTVPSSTWPSETVTCNVAHPASSTKVDKKIVPRDCGCKPCICTVPEVSSVFIFPPKPKDVLTITLTPKVTCVVVDISKDDPEVQFSWFVDDVEVHTAQTQPREEQFNSTFRSVSELPIMHQDWLNGKEFKCRVNSAAFPAPIEKTISKTKGRPKAPQVYTIPPPKEQMAKDKVSLTCMITDFFPEDITVEWQWNGQPAENYKNTQPIMDTDGSYFVYSKLNVQKSNWEAGNTFTCSVLHEGLHNHHTEKSLSHSPGK

SEQ ID NO: 10 - protein, 214 aa, Murine monoclonal antibody (LC of mAb A)
DIVMTQSHKFMSTSVGDRVSITCKASQDVSTAVAWYQQKPGQSPKLLIYSASYRYTGVPDRFTGSGSGTDFTFTISSVQAEDLAVYYCQQHYSSPHTFGGGTKLETKRADAAPTVSIFPPSSEQLTSGGASVVCFLNNFYPKDINVKWKIDGSERQNGVLNSWTDQDSKDSTYSMSSTLTLTKDEYERHNSYTCEATHKTSTSPIVKSFNRNEC

SEQ ID NO: 11 - protein, 455 aa, Murine monoclonal antibody (HC of mAb B)
QVQLKESGPGLLAPSQSLSITCTVSGFSLTGHGVNWVRQPPGKGLEWLGIIWADGTTNYNSALKSRLSISKDNSKSQVFLKMNSLQTDDTASYYCAREGDISGYYFDYWGQGTTLTVSSAKTTPPSVYPLAPGCGDTTGSSVTLGCLVKGYFPESVTVTWNSGSLSSSVHTFPALLQSGLYTMSSSVTVPSSTWPSQTVTCSVAHPASSTTVDKKLEPSGPISTINPCPPCKECHKCPAPNLEGGPSVFIFPPNIKDVLMISLTPKVTCVVVDVSEDDPDVQISWFVNNVEVHTAQTQTHREDYNSTIRVVSTLPIQHQDWMSGKEFKCKVNNKDLPSPIERTISKIKGLVRAPQVYILPPPAEQLSRKDVSLTCLVVGFNPGDISVEWTSNGHTEENYKDTAPVLDSDGSYFIYSKLNMKTSKWEKTDSFSCNVRHEGLKNYYLKKTISRSPGK

SEQ ID NO: 12 - protein, 214 aa, Murine monoclonal antibody (LC of mAb B)
DVQMTQTTSSLSASLGDRVTITCRPSQDINNYLSWYQQKPDGTVKLLIYYTSRLHSGVPSRFSGSGSGTDYSLTISNLEQEDFATYFCQQGNTLPPTFGGGTKLEIKRADAAPTVSIFPPSSEQLTSGGASVVCFLNNFYPKDINVKWKIDGSERQNGVLNSWTDQDSKDSTYSMSSTLTLTKDEYERHNSYTCEATHKTSTSPIVKSFNRNEC